European Patent Application EP 4 389 761 A1, published June 26, 2024. Title: 一种抗新型冠状病毒的多肽及其应用. Applicant: 中国科学院微生物研究所. The sequence listing filed with the application follows.

SEQUENCE LISTING (19 sequences)

SEQ ID NO: 1 - protein, 35 aa, synthetic construct
ISGINASVVNIQKEIDRLNEVAKNLNESLIDLQEL

SEQ ID NO: 2 - protein, 35 aa, synthetic construct
ISGINASVVNIQKEIDRLNEVAKNLNESLIDLKEL

SEQ ID NO: 3 - protein, 40 aa, synthetic construct
VDLGDISGINASVVNIQKEIDRLNEVAKNLNESLIDLQEL

SEQ ID NO: 4 - protein, 40 aa, synthetic construct
VKFGDISGINASVVNIKEEIDRLYEVVKNLNESLIDLQEL

SEQ ID NO: 5 - protein, 35 aa, synthetic construct
ISGINASVVNIKEEIDRLNEVAKNLNESLIDLQEL

SEQ ID NO: 6 - protein, 35 aa, synthetic construct
ISGINASVVNIQKEIDRLNEVAKELNESLIDLQEL

SEQ ID NO: 7 - DNA, 105 bp, synthetic construct
  source 1..105: mol_type = other DNA
attagcggcattaacgcctctgtggtgaacattcagaaggagattgacagactgaacgaggtggccaagaacctgaacgagtctctcattgacctgcaggagctg

SEQ ID NO: 8 - DNA, 105 bp
attagcggcattaacgcctctgtggtgaacattcagaaggagattgacagactgaacgaggtggccaagaacctgaacgagtctctcattgacctgaaggagctg

SEQ ID NO: 9 - DNA, 120 bp, synthetic construct
  source 1..120: mol_type = other DNA
gtggacctgggcgacattagcggcattaacgcctctgtggtgaacattcagaaggagattgacagactgaacgaggtggccaagaacctgaacgagtctctcattgacctgcaggagctg

SEQ ID NO: 10 - DNA, 120 bp, synthetic construct
  source 1..120: mol_type = other DNA
gtgaagttcggcgacattagcggcattaacgcctctgtggtgaacattaaggaggagattgacagactgtacgaggtggtgaagaacctgaacgagtctctcattgacctgcaggagctg

SEQ ID NO: 11 - DNA, 105 bp, synthetic construct
  source 1..105: mol_type = other DNA
attagcggcattaacgcctctgtggtgaacattaaggaggagattgacagactgaacgaggtggccaagaacctgaacgagtctctcattgacctgcaggagctg

SEQ ID NO: 12 - DNA, 105 bp, synthetic construct
  source 1..105: mol_type = other DNA
attagcggcattaacgcctctgtggtgaacattcagaaggagattgacagactgaacgaggtggccaaggagctgaacgagtctctcattgacctgcaggagctg

SEQ ID NO: 13 - DNA, 3756 bp, synthetic construct
  source 1..3756: mol_type = other DNA
atgttcgtgttcctggtgctgctgcccctggtgagcagccaatgcgtgaacctgaccacaagaacacagctgccccccgcctacaccaacagcttcacaagaggcgtgtactaccccgacaaggtgttcagaagcagcgtcctccacagcacccaagacctgttcctgcccttcttcagcaacgtgacctggttccacgccatcagcggcaccaacggcaccaagagattcgacaaccccgtgctgcccttcaacgacggcgtgtacttcgctagcaccgagaagagcaacatcatcagaggctggatcttcggcaccaccctggacagcaaaacacagagcctgctgatcgtgaacaacgccacaaacgtggtgatcaaggtgtgcgagtttcagttctgcaacgaccccttcctgggcgtgtaccacaagaacaacaagagctggatggagagcgagttccgggtgtacagcagcgccaacaactgcaccttcgagtacgtgagccaacccttcctgatggacctggagggcaagcaaggcaattttaagaacctgagagagttcgtgttcaagaacatcgacggctacttcaagatctacagcaagcacacccccatcaacctggtgagagacctgccccaaggcttcagcgccctggagcccctggtggacctgcccatcggcatcaacatcacaagatttcagaccctgctggccctgcacagaagctatctgacccccggcgacagcagcagcggctggaccgccggcgccgccgcttactacgtgggctacctgcagcctagaaccttcctgctgaagtacaacgagaacggcacaatcaccgacgccgtcgactgcgccctggaccccctgagcgagaccaagtgcaccctgaagagcttcaccgtggagaagggcatctatcagacaagcaacttcagagtgcagcccaccgagagcatcgtgagattccccaacatcaccaacctgtgccccttcggcgaggtgttcaacgccacaagattcgctagcgtgtacgcctggaacagaaagagaatcagcaactgcgtggccgactacagcgtgctgtacaacagcgctagcttcagcaccttcaagtgctacggcgtcagccccaccaagctgaacgacctgtgcttcaccaacgtgtacgccgacagcttcgtgatcagaggcgacgaggtgagacagatcgcccccgggcagaccggcaagatcgccgactacaactacaagctgcccgacgacttcaccggctgcgtgatcgcctggaacagcaacaacctggactccaaggtgggcggcaactacaactacctgtacagactgttcagaaagagcaacctgaagcccttcgagagagacatcagcaccgagatctaccaagccggcagcaccccctgcaacggcgtggagggcttcaactgctacttccccctgcagagctacggctttcagcccacctacggcgtgggctatcagccctacagagtggtcgtgctgagcttcgagctgctgcacgcccccgccaccgtgtgcggccccaagaagagcaccaacctggtgaagaacaagtgcgtgaacttcaacttcaacggcctcaccgggaccggcgtgctgaccgagagcaacaagaagttcctgcctttccaacagttcggcagagacatcgacgacaccaccgacgccgtcagagaccctcagaccctggagatcctggacatcacaccctgcagcttcggcggcgtgagcgtgatcacccccggcaccaacacaagcaaccaagtggccgtgctgtaccaaggcgtgaactgcaccgaggtgcccgtggccatccacgccgatcagctgacccccacctggagagtgtacagcaccggcagcaacgtgtttcagacaagagccggctgcctgatcggcgccgagcacgtgaacaacagctacgagtgcgacatccccatcggcgccggcatctgcgctagctatcagacacagaccaacagccacagaagagctagaagcgtggctagccaaagcatcatcgcctacaccatgagcctgggcgccgagaacagcgtggcctacagcaacaacagcatcgccatccccaccaacttcaccatcagcgtgaccaccgaaatcctgcctgtgagcatgaccaagacaagcgtggactgcaccatgtacatctgcggcgacagcaccgagtgcagcaacctgctcctgcagtacggcagcttctgcattcagctgaacagagccctgaccggcatcgccgtggagcaagacaagaacacccaagaggtgttcgcccaagtgaagcagatctacaagaccccccccatcaaggacttcggcggcttcaacttcagccaaatcctgcctgaccctagcaagcctagcaagagaagcttcatcgaggacctgctgttcaacaaggtgaccctggccgacgccggcttcatcaagcagtacggcgactgcctgggcgacatcgccgctagagacctgatctgcgctcagaagttcaacggcctgaccgtgctgccccccctgctgaccgacgagatgatcgctcagtacacaagcgccctgctcgctggcaccatcacaagcgggtggaccttcggcgccggggccgccctgcagatccccttcgccatgcagatggcctacagattcaacggcatcggcgtgacacagaacgtgctgtacgagaatcagaagctgatcgccaatcagttcaacagcgccatcggcaagatccaagacagcctgagcagcaccgctagcgccctgggcaagctgcaagacgtggtgaatcagaacgcccaagccctgaacaccctggtgaagcagctgagcagcaacttcggcgccatcagcagcgtgctgaacgacatcctggctagactggacaaggtggaggccgaggtgcagatcgatagactgatcaccggcagactgcagagcctgcagacctacgtgacacagcagctgatcagagccgccgagatcagagctagcgccaacctggccgccaccaagatgagcgagtgcgtgctggggcagagcaagagagtggacttctgcggcaagggctaccacctgatgagcttccctcagagcgccccccacggcgtggtgttcctgcacgtgacctacgtgcccgcccaagagaagaacttcaccaccgcccccgccatctgccacgacggcaaggcccacttccctagagagggcgtgttcgtgagcaacggcacccactggttcgtgacacagagaaacttctacgagcctcagatcatcaccacccacaacaccttcgtgagcggcaactgcgacgtggtgatcggcatcgtgaacaacaccgtgtacgaccctctgcagcccgagctggacagcttcaaggaggagctggacaagtacttcaagaaccacacaagccccgacgtggacctgggcgacatcagcgggatcaacgctagcgtggtgaacattcagaaggaaatcgacagactgaatgaggtggccaagaacctgaacgagagcctgatcgacctgcaagagctgggcaagtacgagcagtacatcaagtggccctggtacatctggctgggcttcatcgccggcctgatcgccatcgtgatggtgaccatcatgctgtgctgcatgacaagctgctgctcctgtctgaaggggtgctgcagctgcggcagctgctgcaag

SEQ ID NO: 14 - DNA, 3765 bp, synthetic construct
  source 1..3765: mol_type = other DNA
atgttcgtgttcctcgtgctcctgcctctggtgtctagccagtgcgtgaacctgaccacacggacccagctccctcccgcctacacaaactctttcacccggggcgtgtactaccccgacaaggtgttccggtctagcgtgctccactctacacaggacctgttcctccctttcttcagcaacgtgacatggttccacgccatccacgtgtctggcacaaacggcacaaagcggttcgacaaccccgtgctccctttcaacgacggcgtgtacttcgccagcaccgagaagtctaacattatccggggctggattttcggcaccacactcgactctaagacacagtccctcctgattgtgaacaacgccacaaacgtggtgattaaggtgtgcgagttccagttctgcaacgaccctttcctgggcgtgtactaccacaagaacaacaagtcttggatggagtctgagttcagagtgtactctagcgccaacaactgcaccttcgagtacgtgtcccagcctttcctcatggacctggagggcaagcagggcaacttcaagaacctgagagagttcgtgttcaagaacattgacggctacttcaagatttactctaagcacaccccaattaacctcgtgagggacctccctcagggcttctccgccttagaaccactggtggacctccctattggcattaacatcacacgcttccagacactgctcgccctccaccggtcttacctgaccccaggcgactctagctctggctggacagccggcgccgccgcctactacgtgggctacctgcagcctaggaccttcctcctgaagtacaacgagaacggcacaattaccgacgccgtggactgcgccctggacccactgtccgagacaaagtgcacactgaagtccttcacagtggagaagggcatttaccagacatctaacttccgggtgcagcctacagagtctattgtgcggttcccaaacatcacaaacctgtgccctttcggcgaggtgttcaacgccacccggttcgcctctgtgtacgcctggaaccggaagcggatctctaactgcgtggccgactactccgtgctgtacaactccgcctctttctctacattcaagtgctacggcgtgtcccctacaaagctgaacgacctgtgcttcaccaacgtgtacgccgactctttcgtgattagaggcgacgaggtgaggcagattgcccccggccagacaggcaagatcgccgactacaactacaagctgcccgacgacttcacaggctgcgtgatcgcctggaactctaacaacctggactctaaggtgggcggcaactacaactacctgtacagactgttccggaagtctaacctgaagccattcgagagggacattagcaccgagatttaccaggccggctctaccccatgcaacggcgtggagggcttcaactgctacttcccactgcagtcctacggcttccagcctacaaacggcgtgggctaccagccttaccgggtggtggtgctgtctttcgagctgctccacgcccccgccacagtgtgcggcccaaagaagagcacaaacctcgtgaagaacaagtgcgtgaacttcaacttcaacggcctcacaggcacaggcgtgctcaccgagtctaacaagaagttcctccctttccagcagttcggccgcgacattgccgacaccaccgacgccgtgcgggaccctcagacactggaaattctcgacatcaccccttgcagcttcggcggcgtgtccgtgatcaccccaggcacaaacacatctaaccaggtggccgtgctgtaccagggcgtgaactgcaccgaggtgccagtggccatccacgccgaccagctcaccccaacatggagggtgtacagcacaggctctaacgtgttccaaacccgggccggctgcctcattggcgccgagcacgtgaacaactcttacgagtgcgacatccctattggcgccggcatttgcgcctcttaccagacccagacaaactctccacggagagcccggtctgtggcctctcagagcattattgcctacaccatgtctctgggcgccgagaactctgtggcctactctaacaactctattgccatccctacaaacttcacaatttctgtgaccaccgagattctcccagtgtctatgaccaagacatctgtggactgcaccatgtacatttgcggcgactccaccgagtgctctaacctcctgctccagtacggctctttctgcacccagctcaaccgcgccctgacaggcatcgccgtggagcaggacaagaacacccaggaggtgttcgcccaggtgaagcagatttacaagacccccccaattaaggacttcggcggcttcaacttctctcagattctccccgacccatccaagcctagcaagcggtccttcattgaggacctcctgttcaacaaggtgacactggccgacgccggcttcattaagcagtacggcgactgcctgggcgacattgccgcccgggacctgatttgcgcccagaagttcaacggcctcacagtgctccccccactgctcaccgacgagatgattgcccagtacacatctgccctcctggccggcacaattacatctggctggaccttcggcgccggcgccgccctgcagatccctttcgccatgcagatggcctaccgcttcaacggcatcggcgtgacacagaacgtgctgtacgagaaccagaagctgatcgccaaccagttcaacagcgccattggcaagattcaggactctctgagcagcacagccagcgccctgggcaagctgcaggacgtggtgaaccagaacgcccaggccctgaacacactggtgaagcagctgtcttctaacttcggcgccatttctagcgtgctgaacgacattctgtcgcggctggacaaggtggaggccgaggtgcagattgacaggctcatcacaggcagactgcagtctctgcagacatacgtgacccagcagctgattagagccgccgagattagagcctccgccaacctggccgccaccaagatgagcgagtgcgtgctcggccagtctaagcgggtggacttctgcggcaagggctaccacctcatgtctttccctcagtccgcccctcacggcgtggtgttcctccacgtgacatacgtgcccgcccaggagaagaacttcaccacagcccccgccatttgccacgacggcaaggcccacttccctagggagggcgtgttcgtgtctaacggcacccactggttcgtgacccagcggaacttctacgagcctcagattattaccacagacaacacattcgtgagcggcaactgcgacgtggtgattggcattgtgaacaacacagtgtacgacccactgcagcctgagttggactctttcaaggaggaactcgacaagtacttcaagaaccacacatctcctgacgtggacctgggcgacattagcggcattaacgcctctgtggtgaacattcagaaggagattgacagactgaacgaggtggccaaggagctgaacgagtctctcattgacctgcaggagctgggcaagtacgagcagtacattaagtggccttggtacatttggctgggcttcattgccggcctgatcgccattgtgatggtgaccatcatgctgtgctgcatgacatcttgctgcagctgcctgaagggctgctgctcttgcggctcttgctgcaag

SEQ ID NO: 15 - DNA, 3756 bp, synthetic construct; identical to SEQ ID NO: 13
  source 1..3756: mol_type = other DNA

SEQ ID NO: 16 - DNA, 3756 bp, synthetic construct
  source 1..3756: mol_type = other DNA
atgttcgtgttcctggtgctgctgcccctggtgagcagccaatgcgtgaacttcaccacacggacccagctccctcccgcctacacaaactctttcacccggggcgtgtactaccccgacaaggtgttccggtctagcgtgctccactctacacaggacctgttcctccctttcttcagcaacgtgacatggttccacgccatccacgtgtctggcacaaacggcacaaagcggttcgccaaccccgtgctccctttcaacgacggcgtgtacttcgccagcaccgagaagtctaacattatccggggctggattttcggcaccacactcgactctaagacacagtccctcctgattgtgaacaacgccacaaacgtggtgattaaggtgtgcgagttccagttctgcaacgaccctttcctgggcgtgtactaccacaagaacaacaagtcttggatggagtctgagttcagagtgtactctagcgccaacaactgcaccttcgagtacgtgtcccagcctttcctcatggacctggagggcaagcagggcaacttcaagaacctgagagagttcgtgttcaagaacattgacggctacttcaagatttactctaagcacaccccaattaacctcgtgaggggcctccctcagggcttctccgccttagaaccactggtggacctccctattggcattaacatcacacgcttccagacactgcacatctcttacctgaccccaggcgactctagctctggctggacagccggcgccgccgcctactacgtgggctacctgcagcctaggaccttcctcctgaagtacaacgagaacggcacaattaccgacgccgtggactgcgccctggacccactgtccgagacaaagtgcacactgaagtccttcacagtggagaagggcatttaccagacatctaacttccgggtgcagcctacagagtctattgtgcggttcccaaacatcacaaacctgtgccctttcggcgaggtgttcaacgccacccggttcgcctctgtgtacgcctggaaccggaagcggatctctaactgcgtggccgactactccgtgctgtacaactccgcctctttctctacattcaagtgctacggcgtgtcccctacaaagctgaacgacctgtgcttcaccaacgtgtacgccgactctttcgtgattagaggcgacgaggtgaggcagattgcccccggccagacaggcaacatcgccgactacaactacaagctgcccgacgacttcacaggctgcgtgatcgcctggaactctaacaacctggactctaaggtgggcggcaactacaactacctgtacagactgttccggaagtctaacctgaagccattcgagagggacattagcaccgagatttaccaggccggctctaccccatgcaacggcgtgaagggcttcaactgctacttcccactgcagtcctacggcttccagcctacatacggcgtgggctaccagccttaccgggtggtggtgctgtctttcgagctgctccacgcccccgccacagtgtgcggcccaaagaagagcacaaacctcgtgaagaacaagtgcgtgaacttcaacttcaacggcctcacaggcacaggcgtgctcaccgagtctaacaagaagttcctccctttccagcagttcggccgcgacattgccgacaccaccgacgccgtgcgggaccctcagacactggaaattctcgacatcaccccttgcagcttcggcggcgtgtccgtgatcaccccaggcacaaacacatctaaccaggtggccgtgctgtaccagggcgtgaactgcaccgaggtgccagtggccatccacgccgaccagctcaccccaacatggagggtgtacagcacaggctctaacgtgttccagacccgggccggctgcctcattggcgccgagcacgtgaacaactcttacgagtgcgacatccctattggcgccggcatttgcgcctcttaccagacccagacaaactctccacggagagcccggtctgtggcctctcagagcattattgcctacaccatgtctctgggcgtggagaactctgtggcctactctaacaactctattgccatccctacaaacttcacaatttctgtgaccaccgagattctcccagtgtctatgaccaagacatctgtggactgcaccatgtacatttgcggcgactccaccgagtgctctaacctcctgctccagtacggctctttctgcacccagctcaaccgcgccctgacaggcatcgccgtggagcaggacaagaacacccaggaggtgttcgcccaggtgaagcagatttacaagacccccccaattaaggacttcggcggcttcaacttctctcagattctccccgacccatccaagcctagcaagcggtccttcattgaggacctcctgttcaacaaggtgacactggccgacgccggcttcattaagcagtacggcgactgcctgggcgacattgccgcccgggacctgatttgcgcccagaagttcaacggcctcacagtgctccccccactgctcaccgacgagatgattgcccagtacacatctgccctcctggccggcacaattacatctggctggaccttcggcgccggcgccgccctgcagatccctttcgccatgcagatggcctaccgcttcaacggcatcggcgtgacacagaacgtgctgtacgagaaccagaagctgatcgccaaccagttcaacagcgccattggcaagattcaggactctctgagcagcacagccagcgccctgggcaagctgcaggacgtggtgaaccagaacgcccaggccctgaacacactggtgaagcagctgtcttctaacttcggcgccatttctagcgtgctgaacgacattctgtcgcggctggacaaggtggaggccgaggtgcagattgacaggctcatcacaggcagactgcagtctctgcagacatacgtgacccagcagctgattagagccgccgagattagagcctccgccaacctggccgccaccaagatgagcgagtgcgtgctcggccagtctaagcgggtggacttctgcggcaagggctaccacctcatgtctttccctcagtccgcccctcacggcgtggtgttcctccacgtgacatacgtgcccgcccaggagaagaacttcaccacagcccccgccatttgccacgacggcaaggcccacttccctagggagggcgtgttcgtgtctaacggcacccactggttcgtgacccagcggaacttctacgagcctcagattattaccacagacaacacattcgtgagcggcaactgcgacgtggtgattggcattgtgaacaacacagtgtacgacccactgcagcctgagttggactctttcaaggaggaactcgacaagtacttcaagaaccacacatctcctgacgtggacctgggcgacattagcggcattaacgcctctgtggtgaacattcagaaggagattgacagactgaacgaggtggccaagaacctgaacgagtctctcattgacctgcaggagctgggcaagtacgagcagtacattaagtggccttggtacatttggctgggcttcattgccggcctgatcgccattgtgatggtgaccatcatgctgtgctgcatgacatcttgctgcagctgcctgaagggctgctgctcttgcggctcttgctgcaag

SEQ ID NO: 17 - DNA, 3765 bp, synthetic construct; identical to SEQ ID NO: 14
  source 1..3765: mol_type = other DNA

SEQ ID NO: 18 - DNA, 3765 bp, synthetic construct
  source 1..3765: mol_type = other DNA
atgttcgtgttcctggtgctgctgcccctggtgagcagccaatgcgtgaacctgaccacaagaacacagctgccccccgcctacaccaacagcttcacaagaggcgtgtactaccccgacaaggtgttcagaagcagcgtgctgcactccacccaagacctgttcctgcccttcttcagcaacgtgacctggttccacgccatccacgtgagcggcaccaacggcaccaagagattcgacaaccccgtgctgcccttcaacgacggcgtgtacttcgctagcaccgagaagagcaacatcatcagaggctggatcttcggcaccaccctcgatagcaagacacagagcctgctgatcgtgaataatgctaccaacgtggtgatcaaggtgtgcgagtttcagttctgcaacgaccccttcctggacgtgtactaccacaagaacaacaagagctggatgaagagcgagttcagagtgtacagcagcgctaacaactgcaccttcgagtacgtgagccaacccttcctgatggacctggagggcaagcaaggcaacttcaagaacctgagagagttcgtgttcaagaacatcgacggctacttcaagatctacagcaagcacacccccatcaacctggtgagagacctgccccaaggcttcagcgccctggagcccctggtggacctgcccatcggcatcaacatcacaagatttcagaccctgctggccctgcacagatcctacctcacccccggcgatagcagcagcgggtggacagccggcgctgccgcctactacgtgggctacctgcagcctagaaccttcctgctgaagtacaacgagaacggcaccattaccgacgctgtggactgtgccctggaccccctgagcgagaccaagtgcaccctgaagagcttcaccgtggagaagggcatctatcagacaagcaacttcagagtgcagcccaccgagagcatcgtgagattccccaacatcaccaacctgtgccccttcggcgaggtgttcaacgccacaagattcgctagcgtgtacgcctggaatagaaagagaatcagcaactgcgtggccgactacagcgtgctgtacaacagcgctagcttcagcaccttcaaatgctatggcgtgagccccaccaagctgaacgacctgtgcttcaccaacgtgtacgccgacagcttcgtgatcagaggcgacgaggtgagacagatcgcccccgggcagaccggcaagatcgccgattacaactacaaactgcccgacgacttcaccggctgcgtgatcgcctggaacagcaacaacctggacagcaaggtcggcggcaactacaactacagatacagactgttcagaaagagcaacctgaagcccttcgagagagacatcagcaccgagatctaccaagccggcagcaccccctgcaacggcgtgcaaggcttcaactgctacttccccctgcagagctacggctttcagcccaccaacggcgtgggctatcagccctacagagtggtcgtgctgagcttcgagctgctgcacgctcccgccaccgtctgcggccccaagaagtccaccaacctcgtgaagaacaagtgcgtgaacttcaactttaacggcctgaccgggaccggcgtgctgaccgagagcaacaagaagtttctgcccttccaacagttcggcagagacatcgccgacaccaccgacgccgtgagagaccctcagaccctggagatcctggacatcaccccttgtagcttcggcggcgtgagcgtgatcacccccggcaccaacacaagcaaccaagtggccgtgctgtaccaaggcgtgaactgcaccgaggtgcccgtggccatccacgccgatcagctgacccccacctggagagtctacagcaccggcagcaacgtgtttcagacaagagccggctgcctgatcggcgccgagcacgtgaacaacagctacgagtgcgacatccccatcggcgccggcatctgcgctagctatcagacacagaccaacagcagacggagagctagaagcgtggctagccaaagcatcatcgcctacaccatgagcctgggcgccgagaacagcgtggcctacagcaacaacagcatcgccatccccaccaacttcaccatcagcgtgaccaccgagatcctgcccgtcagcatgaccaagacaagcgtggactgcaccatgtacatctgcggcgacagcaccgagtgcagcaacctgctcctgcagtacggcagcttctgcacacagctgaacagagccctgaccggcatcgccgtggagcaagacaagaacacccaagaggtgttcgcccaagtgaagcagatctacaagaccccccccatcaaggacttcggcggcttcaacttcagccaaatcctccccgatcctagcaagcctagcaagagaagcttcatcgaggacctgctgttcaacaaggtgaccctggccgacgccggcttcatcaagcagtacggcgactgcctgggcgacatcgccgctagagacctgatctgcgctcagaagtttaacggcctgaccgtgctcccccccctgctgaccgacgagatgatcgctcagtacacaagcgccctgctggccggcaccatcacaagcggctggacatttggcgccggcgccgctctgcagatccccttcgccatgcagatggcctacagattcaacggcatcggcgtgacacagaacgtgctgtacgagaatcagaagctgatcgccaatcagttcaacagcgccatcggcaagatccaagacagcctgagcagcaccgctagcgccctgggcaagctgcaagacgtggtgaatcagaacgcccaagccctgaacaccctggtgaagcagctgagcagcaacttcggcgccatcagcagcgtgctgaacgatatcctgagcagactggacaaggtggaggccgaggtgcagatcgatagactgattaccggcagactgcagagcctgcagacctacgtgacacagcagctgatcagagccgccgagatcagagctagcgccaacctggccgccaccaagatgagcgagtgcgtgctggggcagagcaagagagtggacttctgcggcaagggctaccacctgatgagcttccctcagagcgccccccacggcgtggtgttcctgcacgtgacctacgtgcccgcccacgaaaagaacttcacaaccgcccctgccatctgccacgacggcaaggcccacttccctagagagggcgtgttcgtgagcaacggcaccgactggttcgtgacacagagaaacttctacgagcctcagatcatcaccaccgacaacaccttcgtgagcggcaactgcgacgtggtgatcggcatcgtgaacaacaccgtgtacgaccctctgcagcccgagctggacagcttcaaggaggagctggacaagtacttcaagaatcacacaagccccgacgtggacctgggggacatcagcggcatcaacgctagcgtggtgaacattcagaaggagatcgacagactgaacgaagtggccaagaacctgaacgagagcctgatcgacctgcaagagctgggcaagtacgagcagtacatcaagtggccctggtacatctggctgggcttcatcgccggcctgatcgccatcgtgatggtgaccatcatgctgtgctgcatgacaagctgctgcagctgcctgaagggctgctgctcctgcggcagctgctgcaag

SEQ ID NO: 19 - DNA, 3759 bp, synthetic construct
  source 1..3759: mol_type = other DNA
atgttcgtgttcctcgtgctcctgcctctggtgtctagccagtgcgtgaacctgagaacacggacccagctccctcccgcctacacaaactctttcacccggggcgtgtactaccccgacaaggtgttccggtctagcgtgctccactctacacaggacctgttcctccctttcttcagcaacgtgacatggttccacgccatccacgtgtctggcacaaacggcacaaagcggttcgacaaccccgtgctccctttcaacgacggcgtgtacttcgccagcaccgagaagtctaacattatccggggctggattttcggcaccacactcgactctaagacacagtccctcctgattgtgaacaacgccacaaacgtggtgattaaggtgtgcgagttccagttctgcaacgaccctttcctggacgtgtactaccacaagaacaacaagtcttggatggagtctggcgtgtactctagcgccaacaactgcaccttcgagtacgtgtcccagcctttcctcatggacctggagggcaagcagggcaacttcaagaacctgagagagttcgtgttcaagaacattgacggctacttcaagatttactctaagcacaccccaattaacctcgtgagggacctccctcagggcttctccgtgttagaaccactggtggacctccctattggcattaacatcacacgcttccagacactgctcgccctccaccggtcttacctgaccccaggcgactctagctctggctggacagccggcgccgccgcctactacgtgggctacctgcagcctaggaccttcctcctgaagtacaacgagaacggcacaattaccgacgccgtggactgcgccctggacccactgtccgagacaaagtgcacactgaagtccttcacagtggagaagggcatttaccagacatctaacttccgggtgcagcctacagagtctattgtgcggttcccaaacatcacaaacctgtgccctttcggcgaggtgttcaacgccacccggttcgcctctgtgtacgcctggaaccggaagcggatctctaactgcgtggccgactactccgtgctgtacaactccgcctctttctctacattcaagtgctacggcgtgtcccctacaaagctgaacgacctgtgcttcaccaacgtgtacgccgactctttcgtgattagaggcgacgaggtgaggcagattgcccccggccagacaggcaagatcgccgactacaactacaagctgcccgacgacttcacaggctgcgtgatcgcctggaactctaacaacctggactctaaggtgggcggcaactacaactacagatacagactgttccggaagtctaacctgaagccattcgagagggacattagcaccgagatttaccaggccggctctaagccatgcaacggcgtggagggcttcaactgctacttcccactgcagtcctacggcttccagcctacaaacggcgtgggctaccagccttaccgggtggtggtgctgtctttcgagctgctccacgcccccgccacagtgtgcggcccaaagaagagcacaaacctcgtgaagaacaagtgcgtgaacttcaacttcaacggcctcacaggcacaggcgtgctcaccgagtctaacaagaagttcctccctttccagcagttcggccgcgacattgccgacaccaccgacgccgtgcgggaccctcagacactggaaattctcgacatcaccccttgcagcttcggcggcgtgtccgtgatcaccccaggcacaaacacatctaaccaggtggccgtgctgtaccagggcgtgaactgcaccgaggtgccagtggccatccacgccgaccagctcaccccaacatggagggtgtacagcacaggctctaacgtgttccagacccgggccggctgcctcattggcgccgagcacgtgaacaactcttacgagtgcgacatccctattggcgccggcatttgcgcctcttaccagacccagacaaactctagacggagagcccggtctgtggcctctcagagcattattgcctacaccatgtctctgggcgccgagaactctgtggcctactctaacaactctattgccatccctacaaacttcacaatttctgtgaccaccgagattctcccagtgtctatgaccaagacatctgtggactgcaccatgtacatttgcggcgactccaccgagtgctctaacctcctgctccagtacggctctttctgcacccagctcaaccgcgccctgacaggcatcgccgtggagcaggacaagaacacccaggaggtgttcgcccaggtgaagcagatttacaagacccccccaattaaggacttcggcggcttcaacttctctcagattctccccgacccatccaagcctagcaagcggtccttcattgaggacctcctgttcaacaaggtgacactggccgacgccggcttcattaagcagtacggcgactgcctgggcgacattgccgcccgggacctgatttgcgcccagaagttcaacggcctcacagtgctccccccactgctcaccgacgagatgattgcccagtacacatctgccctcctggccggcacaattacatctggctggaccttcggcgccggcgccgccctgcagatccctttcgccatgcagatggcctaccgcttcaacggcatcggcgtgacacagaacgtgctgtacgagaaccagaagctgatcgccaaccagttcaacagcgccattggcaagattcaggactctctgagcagcacagccagcgccctgggcaagctgcagaacgtggtgaaccagaacgcccaggccctgaacacactggtgaagcagctgtcttctaacttcggcgccatttctagcgtgctgaacgacattctgtcgcggctggacaaggtggaggccgaggtgcagattgacaggctcatcacaggcagactgcagtctctgcagacatacgtgacccagcagctgattagagccgccgagattagagcctccgccaacctggccgccaccaagatgagcgagtgcgtgctcggccagtctaagcgggtggacttctgcggcaagggctaccacctcatgtctttccctcagtccgcccctcacggcgtggtgttcctccacgtgacatacgtgcccgcccaggagaagaacttcaccacagcccccgccatttgccacgacggcaaggcccacttccctagggagggcgtgttcgtgtctaacggcacccactggttcgtgacccagcggaacttctacgagcctcagattattaccacagacaacacattcgtgagcggcaactgcgacgtggtgattggcattgtgaacaacacagtgtacgacccactgcagcctgagttggactctttcaaggaggaactcgacaagtacttcaagaaccacacatctcctgacgtggacctgggcgacattagcggcattaacgcctctgtggtgaacattcagaaggagattgacagactgaacgaggtggccaagaacctgaacgagtctctcattgacctgcaggagctgggcaagtacgagcagtacattaagtggccttggtacatttggctgggcttcattgccggcctgatcgccattgtgatggtgaccatcatgctgtgctgcatgacatcttgctgcagctgcctgaagggctgctgctcttgcggctcttgctgcaag